European Patent Application EP 4 632 072 A1, published October 15, 2025. Title: A microorganism introduced with exogenous soluble pyridine nucleotide transhydrogenase, and method for producing L-tryptophan using the same. Applicant: CJ CheilJedang Corporation. The sequence listing filed with the application follows.

SEQUENCE LISTING (37 sequences)

SEQ ID NO: 1 - protein, 464 aa, Pseudomonas aeruginosa
MAVYNYDVVILGTGPAGEGAAMNASKYGRKLAVVDSRRVVGGNCTHLGTIPSKALRHSVKQIIEFNTNPMFRQIGEPRWFSFPDVLKSADRVISKQVASRTGYYARNRIDMFTGTASFVDERTVEVVTPSGAVERLVADQFVIATGSRPYRPSDINFNHPRVYDSDTILSLSHTPRRLIIYGAGVIGCEYASIFSGLGVLVDLIDTRDQLLSFLDDEISDALSYHLRNNNVLIRHNEEYERVEGLDNGVILHLKSGKKIKADALLWCNGRTGNTDKLGLENVGIKVNSRGQIEVDENYRTSVSNIFAAGDVIGWPSLASAAYDQGRSAAGNIVESDSWRFVNDVPTGIYTIPEISSIGKNESELTAAKIPYEVGKAFFKGMARAQISNEPVGMLKILFHRETLEILGVHCFGDQASEIVHIGQAIMNQPGELNTLKYFVNTTFNYPTMAEAYRVAAFDGLNRLF

SEQ ID NO: 2 - DNA, 1395 bp, Pseudomonas aeruginosa
  source 1..1395: mol_type = genomic DNA
atggctgtctacaactacgacgtggtgattttgggcacgggtccggcgggcgaaggggcggcgatgaacgcctccaagtacggacgcaagctggcggtagtcgacagccgtcgcgtggtcggaggcaactgcacgcacctcggcaccattccttccaaggccctgcgccactcggtgaagcagatcatcgagttcaacaccaacccgatgttccgccagatcggcgagccgcgctggttctccttccccgacgtgctgaagagcgccgaccgggtgatctccaagcaggtcgcttcgcgtaccggctactacgcgcgcaatcgcatcgacatgttcaccggcaccgccagcttcgtcgacgaacgcaccgtcgaagtggtgacgccgagcggcgcggtggagcgcctggtcgccgaccagttcgtgatcgccaccggctcgcgcccgtatcgtccttcggacatcaatttcaaccacccgcgggtctacgacagcgacaccatcctgtccctgagccacaccccgcgccggctgatcatctacggagccggggtgatcggctgcgaatacgcgtcgatcttcagcggcctgggcgtgctggtggacctgatcgatacgcgcgaccagttgctcagcttcctcgatgacgagatttccgatgcgctgagctaccacctgcgcaacaacaacgtgctgatccgccacaacgaggagtacgagcgcgtcgaggggctggacaacggtgtcatcctgcacctgaagtcgggcaagaagatcaaggcggacgcgctgctctggtgcaacggccggaccggcaacaccgacaagctcggcctggagaacgtcggcatcaaggtcaacagccgtggccagatcgaggtggacgagaactaccgcacttcggtgagcaacatcttcgccgccggcgacgtgatcggctggccgagcctggccagcgctgcctacgaccagggccgctcggccgccggcaacatcgtcgagagcgacagctggcgcttcgtcaacgatgtgccgaccggcatctacaccattccggagatcagctcgatcggcaagaacgaaagcgaactgaccgcggcgaagattccctacgaagtgggcaaggcgttcttcaagggcatggcccgggcgcagatttccaacgagccggtgggcatgctgaagatcctgttccatcgcgagaccctggagatcctcggcgtgcactgcttcggcgaccaggcttcggaaatcgtccacatcggtcaggcgatcatgaaccagccgggcgagctgaataccctgaagtacttcgtcaacaccaccttcaactacccgaccatggcggaagcctatcgggtagcggcgttcgacggcctcaaccggcttttttga

SEQ ID NO: 3 - protein, 466 aa, Erwinia amylovora
MQKSYDYDAIVIGSGPGGEGAAMGLVKQGARIAVIERYHNIGGGCTHWGTIPSKALRHAVSRIIEFNQNPLYSDHTRLLRSSFADILKHTENVISQQTHMRQGFYERNHCQIYQGDARFVDANTLEIESHDGSIERLTAEKFVIACGSRPYHPPDVDFSHPRIYDSDSILNLHHEPGHVIIYGAGVIGCEYASIFRGLAVKVDLINTRDRLLAFLDQEMSDSLSYHFWNNGVVIRHNEEFDKVEGVADGVIMHLKSGKKLKADCLLYANGRTGNTDSLFLENVGLEADGRGLLKVNSMYQTAQPHIYAVGDVIGYPSLASAAYDQGRIAAQAMIKGEATAHLIEDIPTGIYTIPEISSVGKTEQQLTAMKVPYEVGRAQFKHLARAQIVGMNVGSLKILFHRETKEILGIHCFGERAAEIIHIGQAIMEQKNGGNTIEYFVNTTFNYPTMAEAYRVAALNGLNRLF

SEQ ID NO: 4 - DNA, 1401 bp, Erwinia amylovora
  source 1..1401: mol_type = genomic DNA
atgcaaaagtcttatgattacgacgccattgtcattggatcaggtcccggcggtgaaggtgccgcaatggggctggtgaaacagggtgcgcgcatcgccgtgattgagcgctatcacaatatcggcggcggttgtacacattgggggaccatcccttcgaaagcgctgcgccacgctgtcagccgtattatcgagttcaaccaaaatcccctctatagcgaccatacacgtcttctgcgttcctctttcgccgacatcctcaagcacaccgaaaatgtgattagccagcaaacccatatgcgccagggcttctatgaacgcaaccactgccagatctatcagggggatgcgcgttttgttgatgccaacaccctcgaaattgaaagccatgacggcagcattgaacggctgacggcggaaaagttcgtcattgcctgtggttctcgtccttatcacccaccggacgtcgatttcagccacccgcgtatctatgacagtgactcgatcctcaatctgcaccatgagccaggccatgtgattatctatggtgccggagtgatcggctgtgaatacgcatctattttccgcgggcttgccgttaaagtcgatttgattaatacccgtgaccgcctgctggcattcctcgaccaggaaatgtcagattctctttcctatcatttctggaataacggggtggtgatccgccataacgaagagttcgacaaggttgaaggagtggctgatggcgtcatcatgcacctgaaatcgggtaaaaagctgaaagctgactgcctgctgtacgccaatggccgtaccggcaataccgattcattgtttctggaaaatgttggactggaagcagacggtcgcggcctgctgaaagtgaacagcatgtaccagacggcacagccgcatatctatgcggtaggtgatgtgattggttacccaagcctggcctcggcagcctacgatcaggggcgtattgccgcacaggcaatgatcaaaggggaagcaaccgcccatctgattgaagatatcccaaccgggatctacaccatcccggaaatcagctccgtcgggaaaaccgagcagcagctgacggcgatgaaagtgccctacgaagtgggccgggcgcagtttaagcaccttgcgcgcgcgcagatcgtcggcatgaacgtcggcagcctgaaaatcctgttccaccgtgaaaccaaagagatccttggcattcactgctttggcgaacgtgccgccgagattattcatatcggtcaggcgatcatggaacagaaaaacggtggcaacacgattgagtacttcgtgaataccacctttaactacccgacaatggcggaagcctaccgggttgcggcgctaaacggcctgaaccggctattttag

SEQ ID NO: 5 - protein, 444 aa, Alteromonas mediterranea
MQLAKAGKKVAVVERYEAVGGGCTHWGTIPSKALRHSVSRLIEYNSSPLFADNHLSKSLTFSDIMRHASGVVKSQTRLRSSFYDRNRVTLFYGEASFVDAHTLEITREDGSKDTVTAAQIAIATGSRPYCPKDIDFNHPRVYNSDTILSLDHDPKSIIIYGAGVIGSEYASIFRGLGVKVDLVNMRDRLLSFLDDEISDALSYHLWNNGVLIRHNETYSSVETLDDSVILNLESGKRMRADCLLFANGRTGNTDTLKLENVGLKADNRGQLRVNENYQTEIDNIYAVGDVIGYPSLASAAYNQGRFAAEAMLGISTHSALVADIPSGIYTIPEISSVGKTEQELTAAKVPYEVGRAQFKHLARAQIASTQTGSLKILFHRETKEILGIHCFGERASEIVHIGQAIMQQKGEGNTIDYFVNTTFNYPTMAEAYRVAAINGLNRIF

SEQ ID NO: 6 - DNA, 1335 bp, Alteromonas mediterranea
  source 1..1335: mol_type = genomic DNA
atgcaacttgccaaggccggtaaaaaagtggctgttgtagagcgctatgaagcggtgggtggaggctgtacgcattggggaaccatcccctcgaaagcgcttcgtcattcagttagccggctcattgagtacaactcatcgcctctgtttgccgataaccatttaagcaagagccttacgttctcagatatcatgcgtcatgccagtggcgttgtgaaaagccaaacacgccttcgctcttccttttacgatagaaaccgggtgacactgttttacggcgaagcaagctttgttgatgcgcatactttagagataacgcgtgaagatggttcaaaagacacggttactgcagcgcaaatagctatcgctactggttcccgtccctactgcccgaaagacatcgattttaatcatccaagggtttataactcagataccattttgtcgttagatcacgaccctaaatccatcataatctacggtgcgggtgttatcggttctgaatatgccagcatttttagagggttaggtgttaaagttgatctggttaacatgcgcgatcgcttactttcatttctagatgatgaaatttccgacgccctgagttaccacttatggaataacggcgttctcattcgccacaacgaaacgtattcatcggtcgaaacgttagatgactctgtgattttaaaccttgaatcaggtaagcgaatgcgagcagactgtttactgtttgctaacgggcgtacgggtaacaccgatacccttaagctggagaatgttggtcttaaagcagacaacagagggcaactgcgcgtaaacgaaaactatcagacagagatagataatatctatgccgtcggtgatgtcattggctaccctagtttagcatcagcggcatataaccaaggccggtttgcagcagaagccatgcttggaataagcactcattcagcgcttgttgccgatatcccttccggtatttacactattccggaaataagctccgtaggcaagacagagcaggagttaacagccgctaaagtgccttatgaagtaggacgagcacagttcaagcatttggctagagcacaaattgcgtccacgcaaaccggtagtcttaagattctctttcatcgtgaaacaaaagaaattttgggcattcactgcttcggagagcgtgcctcagaaattgtgcacatcgggcaagctatcatgcagcaaaaaggtgaaggtaataccattgactacttcgttaataccacatttaactatccgactatggctgaagcctatcgcgttgcagcgataaacggcttgaacaggattttctaa

SEQ ID NO: 7 - protein, 462 aa, Spongiibacter sp. IMCC21906
MAYDYDVVVLGSGPAGESAALNASKHGRTVAVVEAQSLVGGACSHQGTIPSKALRHMVRQAIRFNQTQIFRDLGDPRTLTYPKLLSHAEDVISQQVAMRSRFYYRNNITLIHGQAEFVDAHSIAVLREDGKQSKLTAKQIVIATGSRPYRPADIDFNHPRVYDSDSILKMTNTPRKIIVYGAGVIGCEYASIFSGIGMKVELVNTRDRLLEFLDDEISDALSYHLRYTGVMMRHREEYEKVEADDNGVTLYLKSGKRLHCDALLWCNGRSGNTDNLKLSTIGLEADHRGQLSVNEHYQTAVQDIYAAGDVIGWPSLASAAYDQGRAAAATARGKEHCRFVDDVPTGIYTLPEISSFGLSERELTEEKIPYEVGRAFFKDTARGQISGETVGMLKLLFHVDTLEILGIHCFGAEAAEIIHIGQAIMKQPGDGNTLRYFVNTTFNYPTMAEAYRTAALNGLNRL

SEQ ID NO: 8 - DNA, 1389 bp, Spongiibacter sp. IMCC21906
  source 1..1389: mol_type = genomic DNA
atggcatatgattacgacgttgtggtactgggaagtggtcctgcaggtgaatcggcggccttaaatgccagtaaacatggccgtactgtggcggtggttgaggcgcaatcgctggtcggcggcgcctgttctcatcagggtacgattccctccaaggcacttagacatatggtgcgtcaggctattcgatttaatcaaactcagatttttcgagatttgggtgacccccgaacactgacttaccccaagctgttaagtcatgctgaagatgttatttctcagcaggtggcaatgcgcagccgcttttactaccgcaacaatatcacccttattcacggccaggccgagtttgtcgatgcgcatagcattgcggtattacgtgaggacggcaagcagagcaagctgactgccaagcaaattgtgatcgctactgggtcgaggccttatcgcccagccgatatcgattttaatcacccgcgggtgtatgacagcgacagtattttgaagatgaccaacaccccacgaaaaatcatcgtatacggggccggggtaattggctgtgaatatgcgtcgattttttcgggcattggtatgaaagttgagctggtgaatacccgggatcgcttgttggagtttcttgacgatgaaatttctgacgcccttagttatcacctgcgctataccggtgtgatgatgcggcaccgggaagaatatgagaaggttgaggcagacgataacggcgttaccttgtatctcaaatcgggaaaacgtctgcattgtgacgccttgctttggtgtaatggccgcagtggcaacaccgacaatctcaagttgtcgacgattggccttgaggccgatcatcgcggccagctcagtgtgaatgaacattatcaaaccgccgtacaagacatttacgcggcgggtgacgtgattggttggcccagcctggccagtgcggcttatgaccaaggtagagcggctgcggcgacagcacggggtaaagagcattgccgctttgttgatgatgtgcccaccgggatatacaccttgccagaaatcagttcttttggtttgagtgagcgggagctgactgaagaaaagataccctacgaagtaggccgggcgttttttaaggataccgcccgcgggcaaatcagcggtgaaacggtggggatgttaaagctcttgtttcatgtcgataccttggagattttgggaatccactgttttggggccgaggcggcagaaatcatccatatcggccaggcgattatgaagcagcccggcgacggtaataccctacggtattttgtgaatacgacctttaactatcccaccatggcggaggcttatcgcaccgcggcgcttaatggcttaaatcggttataa

SEQ ID NO: 9 - protein, 471 aa, Amycolatopsis albispora
MSAYDYDLIVIGSGPGGQKAAIAAAKLGKRVAVVDRHDMVGGVCVNTGTIPSKTLREAVHYLTGMSQRELYGASYRVKQDITIADLMARTQHVIGREVEVVRAQLMRNGVHLVSGLGRFTDPHTVAVEGGPRGERTSLTGEYVVIATGTRPARPPEVDFDEARVLDSDEILSLDRIPSSLVVVGAGVIGIEYASMFAALGCRVTVVEQRERMLEFCDPEIVESLKFHLRDLAVTFRFGEKVVDVAVGEHATVTSLASGKRIPAEAVMYSAGRQGMTDALGLEHAGLTADKRGRLAVDDHYRTEVPHIYAVGDVIGFPALAATSMDQGRLAAYHAFGEPANELAALQPIGIYTIPEISYCGATEAELTSSSIPYEIGTARYRELARGQIAGDSYGMLKLLVSTEDRKLLGVHVFGTGATDLVHIGQAVMGCGGTVDYLVDTVFNYPTLSEAYKVAALDATNKIRALARFTTT

SEQ ID NO: 10 - DNA, 1416 bp, Amycolatopsis albispora
  source 1..1416: mol_type = genomic DNA
atgagcgcctatgactacgacctgatcgtgatcggctcgggccccggcgggcagaaggccgccatcgccgcggccaagctcggcaagcgcgtggcggtggtcgaccgccacgacatggtcggcggggtgtgcgtcaacaccggcaccattccgtcgaaaacgctgcgtgaggccgtgcactacctgaccgggatgagccagcgtgagctgtacggggccagctaccgggtcaagcaggacatcaccatcgccgacctgatggcccgcacgcagcacgtgatcgggcgcgaggtcgaggtggtgcgcgcgcagctgatgcgcaacggggtgcacctggtcagcggcctcggccggttcaccgacccgcacaccgtcgcggtcgaaggcggtccgcgtggcgagcggacctcactgaccggtgagtacgtggtgatcgccaccggcacccggccggcgcgcccgccggaggtcgacttcgacgaggcccgcgtgctggactccgacgagatcctgagcctggaccgcatcccgtcttcgctggtcgtggtgggtgccggggtgatcggcatcgagtacgcctcgatgttcgccgcgctgggctgccgggtgaccgtggtcgagcagcgggagcggatgctggagttctgcgacccggagatcgtcgaatcgctgaagttccatctccgggacctggcggtgaccttccggttcggcgagaaggtggtcgacgtggcggtcggcgagcacgccacggtgacgtcgctggccagcgggaagcgcatcccggccgaggcggtgatgtactcggccggtcgccagggcatgaccgacgcgctcggcctggagcacgcgggcctgaccgccgacaagcgcggccgcctcgccgtcgacgaccactaccgcaccgaggtcccgcacatctacgccgtcggtgacgtgatcggcttccccgcgctcgccgcgacttcgatggaccagggcaggctggccgcgtaccacgccttcggcgaaccggcgaacgagctggccgcgctgcagccgatcggcatctacaccattccggagatctcctactgcggcgcgaccgaggccgagctgacgtcttcttcgatcccgtacgagatcggtaccgcccggtaccgcgaactggcccgaggccaaatcgccggcgactcgtatggcatgctcaagctgctggtgtccacagaggaccggaaactgctgggcgtgcacgtcttcggcaccggggccaccgacctggtccacatcggacaagccgtaatgggctgcggcggcacggtcgactacctggtggacaccgtgttcaactacccgacgctgtcggaggcgtacaaggtcgccgcactggacgccaccaacaagatccgcgcactggcccgcttcaccacaacctga

SEQ ID NO: 11 - protein, 464 aa, Azotobacter vinelandii
MAVYNYDVVVIGTGPAGEGAAMNAVKAGRKVAVVDDRPQVGGNCTHLGTIPSKALRHSVRQIMQYNNNPLFRQIGEPRWFSFADVLKSAEQVIAKQVSSRTGYYARNRIDTFFGTASFCDEHTIEVVHLNGMVETLVAKQFVIATGSRPYRPADVDFTHPRIYDSDTILSLGHTPRRLIIYGAGVIGCEYASIFSGLGVLVDLIDNRDQLLSFLDDEISDSLSYHLRNNNVLIRHNEEYERVEGLDNGVILHLKSGKKIKADAFLWSNGRTGNTDKLGLENIGLKANGRGQIQVDEHYRTEVSNIYAAGDVIGWPSLASAAYDQGRSAAGSITENDSWRFVDDVPTGIYTIPEISSVGKTERELTQAKVPYEVGKAFFKGMARAQIAVEKAGMLKILFHRETLEILGVHCFGYQASEIVHIGQAIMNQKGEANTLKYFINTTFNYPTMAEAYRVAAYDGLNRLF

SEQ ID NO: 12 - DNA, 1395 bp, Azotobacter vinelandii
  source 1..1395: mol_type = genomic DNA
atggctgtatataactacgatgtggtggtaatcggcacaggccctgctggcgaaggggcagcgatgaatgccgtgaaggccgggcgcaaggtagcggtcgtggatgatcgcccccaggtcggcggcaactgcacccacctcggaaccattccctccaaggcgctgcgccactcggtgcggcagatcatgcagtacaacaacaatccgctgttccgccagatcggcgagccgcgctggttttccttcgccgatgtcctgaagagcgccgagcaggtcatcgccaagcaggtttcctcgcggaccggctactatgcgcgcaaccgtatcgataccttcttcgggaccgcgagcttctgcgacgagcacaccatcgaggtcgtccacctcaacggtatggtggaaacgctggtggccaagcagttcgtcatcgccaccgggtcgcgtccctaccgcccggccgatgtcgatttcacccatccgcgcatctacgacagcgacaccatcctcagcctcggccacacgccgcgccggttgatcatctacggagcgggggtgatcggctgcgaatatgcctccatcttcagtgggctgggcgtgctggtcgacctcatcgacaaccgcgaccaactgctcagtttcctcgacgacgaaatctccgactcgctcagctaccacctgcgcaacaacaacgtgctgatccgccacaacgaggaatacgagcgtgtcgaaggcctggacaacggggtgatcctgcacctcaagtccggcaagaagatcaaggccgacgccttcctgtggagcaacggccgtaccggcaataccgacaagctgggcctggagaacatcggtctcaaggccaatggtcgcggacagatccaggtcgacgagcactaccgtaccgaagtcagcaacatctatgccgctggtgacgtgatcggctggccgagcctggccagcgccgcctatgaccagggtcgttcggccgcgggcagtatcaccgagaacgatagctggcgtttcgtcgacgacgtgccgaccggcatctacaccattccggagatcagttcggtcggcaagaccgagcgcgaactgacccaggcgaaggttccctacgaggtcggcaaggccttcttcaagggcatggcccgggcacagatcgccgtcgagaaggccggcatgctgaagatcctctttcaccgcgagacgctggaaatcctcggcgtgcactgcttcggctatcaggcttcggaaatcgtccatatcggccaggcgatcatgaaccagaagggcgaggcgaataccctcaagtatttcatcaacaccaccttcaactacccgaccatggccgaggcctaccgggtggcggcctacgacggtctcaatcggcttttttga

SEQ ID NO: 13 - DNA, 33 bp, synthetic construct
  source 1..33: mol_type = other DNA
tcgagctcggtacccgctggttgattgcgttga

SEQ ID NO: 14 - DNA, 33 bp, synthetic construct
  source 1..33: mol_type = other DNA
cacagtgccagtactcccgatagcgtttttcca

SEQ ID NO: 15 - DNA, 33 bp, synthetic construct
  source 1..33: mol_type = other DNA
gctatcgggagtactggcactgtggtttgtttt

SEQ ID NO: 16 - DNA, 33 bp, synthetic construct
  source 1..33: mol_type = other DNA
ctctagaggatcccctctgtatccacgtgttct

SEQ ID NO: 17 - DNA, 36 bp, synthetic construct
  source 1..36: mol_type = other DNA
gaaaggtgcacacatatggctgtctacaactacgac

SEQ ID NO: 18 - DNA, 38 bp, synthetic construct
  source 1..38: mol_type = other DNA
acaaaccacagtgccagttcaaaaaagccggttgaggc

SEQ ID NO: 19 - DNA, 37 bp, synthetic construct
  source 1..37: mol_type = other DNA
aaacgctatcgggagtggcccttccggtttagtgctc

SEQ ID NO: 20 - DNA, 37 bp, synthetic construct
  source 1..37: mol_type = other DNA
gttgtagacagccatatgtgtgcacctttcgatctac

SEQ ID NO: 21 - DNA, 18 bp, synthetic construct
  source 1..18: mol_type = other DNA
tccacatgccgtattctt

SEQ ID NO: 22 - DNA, 19 bp, synthetic construct
  source 1..19: mol_type = other DNA
gttgtcgattgtgtctggt

SEQ ID NO: 23 - DNA, 40 bp, synthetic construct
  source 1..40: mol_type = other DNA
gaaaggtgcacacatatgcaaaagtcttatgattacgacg

SEQ ID NO: 24 - DNA, 39 bp, synthetic construct
  source 1..39: mol_type = other DNA
aaccacagtgccagtctaaaatagccggttcaggccgtt

SEQ ID NO: 25 - DNA, 37 bp, synthetic construct
  source 1..37: mol_type = other DNA
ataagacttttgcatatgtgtgcacctttcgatctac

SEQ ID NO: 26 - DNA, 35 bp, synthetic construct
  source 1..35: mol_type = other DNA
gaaaggtgcacacatatgcaacttgccaaggccgg

SEQ ID NO: 27 - DNA, 40 bp, synthetic construct
  source 1..40: mol_type = other DNA
aaccacagtgccagtttagaaaatcctgttcaagccgttt

SEQ ID NO: 28 - DNA, 37 bp, synthetic construct
  source 1..37: mol_type = other DNA
cttggcaagttgcatatgtgtgcacctttcgatctac

SEQ ID NO: 29 - DNA, 38 bp, synthetic construct
  source 1..38: mol_type = other DNA
gaaaggtgcacacatatggcatatgattacgacgttgt

SEQ ID NO: 30 - DNA, 40 bp, synthetic construct
  source 1..40: mol_type = other DNA
aaccacagtgccagtttataaccgatttaagccattaagc

SEQ ID NO: 31 - DNA, 37 bp, synthetic construct
  source 1..37: mol_type = other DNA
gtaatcatatgccatatgtgtgcacctttcgatctac

SEQ ID NO: 32 - DNA, 35 bp, synthetic construct
  source 1..35: mol_type = other DNA
gaaaggtgcacacatatgagcgcctatgactacga

SEQ ID NO: 33 - DNA, 35 bp, synthetic construct
  source 1..35: mol_type = other DNA
aaccacagtgccagttcaggttgtggtgaagcggg

SEQ ID NO: 34 - DNA, 37 bp, synthetic construct
  source 1..37: mol_type = other DNA
gtcataggcgctcatatgtgtgcacctttcgatctac

SEQ ID NO: 35 - DNA, 39 bp, synthetic construct
  source 1..39: mol_type = other DNA
gaaaggtgcacacatatggctgtatataactacgatgtg

SEQ ID NO: 36 - DNA, 36 bp, synthetic construct
  source 1..36: mol_type = other DNA
aaccacagtgccagttcaaaaaagccgattgagacc

SEQ ID NO: 37 - DNA, 37 bp, synthetic construct
  source 1..37: mol_type = other DNA
gttatatacagccatatgtgtgcacctttcgatctac